European Patent Application EP 4 324 852 A1, published February 21, 2024. Title: ANTI-HUMAN MASP-2 ANTIBODY, PREPARATION METHOD THEREFOR AND APPLICATION THEREOF. Applicant: Shanghai MABGEEK Biotechnology Co., Ltd. The sequence listing filed with the application follows.

SEQUENCE LISTING (80 sequences)

SEQ ID NO: 1 - protein, 120 aa, Mus musculus
QVQLQQSGAELMKPGASVKISCKATGYPFSTYWIEWVKQRPGHGLEWIGEILPGSDNTNYNEKFKGKATFTADTSSNTAYMQLSSLTSEDSAVYYCARRTTATRAWFVYWGQGTLVTVSA

SEQ ID NO: 2 - protein, 113 aa, Mus musculus
DIVMSQSPSSLAVSVGEKVTMSCKSSQSLLYSSNQKNYLAWYQQKPGQSPKLLIYWASTRESGVPDRFTGSGSGTDFTLTISSVRAEDLAVYYCQHYYTYPWTFGGGTNLEIK

SEQ ID NO: 3 - protein, 116 aa, Mus musculus
DVQLVESGGGLVQPGGSRKLSCAASGFTFSNFGIHWVRQAPEKGLEWVAYISSGGSAVFYADTVKGRFTISRDNSKNTLFLQMTSLRSEDTAIYYCAKSDRYFDYWGQGTTLTVSS

SEQ ID NO: 4 - protein, 111 aa, Mus musculus
DIVLTQSPASLAVSLGQRATISCRASQSVSSSSYRYIHWYQQKPGQPPRLLIKYASNLESGVPARFSGSGSGTDFTLNIHPVEEEDTATYYCQHSWETPWTFGGGTKLEIK

SEQ ID NO: 5 - protein, 116 aa, Mus musculus
DVQLVESGGGLVQPGGSRKLSCAASGFTFSSFGMHWVRQAPEKGLEWVAYISSGSSSFFYADTVKGRFTISRDNPKNTLFLQMTSLRSEDTAMYYCARGDRNFDVWGAGTTVTVSS

SEQ ID NO: 6 - protein, 111 aa, Mus musculus
DIVLTQSPASLAVSLGQRATISCRASQSVTSSRYSYMHWFQQKPGQPPNLLIKHASNLESGVPARFSGSGSGTDFTLNIHPVEEDDTATYYCQHSWEVPWTFGGGTKLEIK

SEQ ID NO: 7 - protein, 116 aa, Mus musculus
DVQLQESGPGLVKPSQSLSLTCTVTGYSITSDYAWSWIRQFLRNKLEWMGYISYSGRTSYNPSLKSRISITRDTSKNQFFLQLNSVTTEDTATYFCARLITGGDYWGQGTSVTVSS

SEQ ID NO: 8 - protein, 107 aa, Mus musculus
DIVMTQSQKFMSTSVGDRVSVTCKASQNVGINVVWYQQKPGQSPKALIYSASYRFSGVPDRFTGSGSGTDFTLTISNVQSEDLAEYLCLQYDINPLTFGAGTKLELK

SEQ ID NO: 9 - protein, 114 aa, Mus musculus
DVQLQESGPGLVKPSQSLSLTCTVTGYSITSDYAWNWIRQFPGNKLEWMGYISYSGRTSYNPSLKSRLSITRDTSKNQFFLQLTSVTTEDTATYYCARHYGDFWGQGTTLTVSS

SEQ ID NO: 10 - protein, 107 aa, Mus musculus
DIVMTQSQKFMSTSVGDRVSVTCKASQNVDTNVAWFQQKPGQSPKPLIYSASYRYSGVPDRFTGSGSGTDFTLTISNVQSEDLANYFCQQYNSYPSTFGSGTKLEIK

SEQ ID NO: 11 - protein, 116 aa, Mus musculus
DVQLVESGGGLVQPGGSRKLSCVASGFTFSSFGMHWVRQAPEKGLEWVAYISSGSSSSFYVDTVKGRFTISRDNPKNTLFLQMTSLRSEDTAMYYCARGDRNFEVWGAGTTVTVSS

SEQ ID NO: 12 - protein, 111 aa, Mus musculus
DIVLTQSPASLAVSLGQRATISCRASQSVSSSRYSYMHWFQQKPGQPPNLLIKHASNLESGVPARFSGSGSGTDFTLNIHPVEEEDTATYYCQQSWEVPWTFGGGTKLEIK

SEQ ID NO: 13 - protein, 117 aa, Mus musculus
QVQLQQSGAELAKPGASVKMSCKASGNTFTNYWMHWIKQRPGQGLEWVGYINPNTGYTDFNQKFKDKATLTADKSSTTAYMQLISLTSEDSTVYYCTLQLGRNFDYWGQGTTLTVSS

SEQ ID NO: 14 - protein, 111 aa, Mus musculus
DIVLTQSPASLGVSLGQRATISCRASQSVSSSRSTYIHWYQQKPGQPPKLLIKYSSNLESGVPARFSGGGSGTDFTLNIHPVEAEDTATYYCHQSWEIPYTFGGGTKLEIR

SEQ ID NO: 15 - protein, 5 aa, Mus musculus
TYWIE

SEQ ID NO: 16 - protein, 17 aa, Mus musculus
EILPGSDNTNYNEKFKG

SEQ ID NO: 17 - protein, 11 aa, Mus musculus
RTTATRAWFVY

SEQ ID NO: 18 - protein, 17 aa, Mus musculus
KSSQSLLYSSNQKNYLA

SEQ ID NO: 19 - protein, 7 aa, Mus musculus
WASTRES

SEQ ID NO: 20 - protein, 9 aa, Mus musculus
QHYYTYPWT

SEQ ID NO: 21 - protein, 5 aa, Mus musculus
NFGIH

SEQ ID NO: 22 - protein, 17 aa, Mus musculus
YISSGGSAVFYADTVKG

SEQ ID NO: 23 - protein, 7 aa, Mus musculus
SDRYFDY

SEQ ID NO: 24 - protein, 15 aa, Mus musculus
RASQSVSSSSYRYIH

SEQ ID NO: 25 - protein, 7 aa, Mus musculus
YASNLES

SEQ ID NO: 26 - protein, 9 aa, Mus musculus
QHSWETPWT

SEQ ID NO: 27 - protein, 5 aa, Mus musculus
SFGMH

SEQ ID NO: 28 - protein, 17 aa, Mus musculus
YISSGSSSFFYADTVKG

SEQ ID NO: 29 - protein, 7 aa, Mus musculus
GDRNFDV

SEQ ID NO: 30 - protein, 15 aa, Mus musculus
RASQSVTSSRYSYMH

SEQ ID NO: 31 - protein, 7 aa, Mus musculus
HASNLES

SEQ ID NO: 32 - protein, 9 aa, Mus musculus
QHSWEVPWT

SEQ ID NO: 33 - protein, 6 aa, Mus musculus
SDYAWS

SEQ ID NO: 34 - protein, 16 aa, Mus musculus
YISYSGRTSYNPSLKS

SEQ ID NO: 35 - protein, 7 aa, Mus musculus
LITGGDY

SEQ ID NO: 36 - protein, 11 aa, Mus musculus
KASQNVGINVV

SEQ ID NO: 37 - protein, 7 aa, Mus musculus
SASYRFS

SEQ ID NO: 38 - protein, 9 aa, Mus musculus
LQYDINPLT

SEQ ID NO: 39 - protein, 6 aa, Mus musculus
SDYAWN

SEQ ID NO: 40 - protein, 16 aa, Mus musculus
YISYSGRTSYNPSLKS

SEQ ID NO: 41 - protein, 5 aa, Mus musculus
HYGDF

SEQ ID NO: 42 - protein, 11 aa, Mus musculus
KASQNVDTNVA

SEQ ID NO: 43 - protein, 7 aa, Mus musculus
SASYRYS

SEQ ID NO: 44 - protein, 9 aa, Mus musculus
QQYNSYPST

SEQ ID NO: 45 - protein, 5 aa, Mus musculus
SFGMH

SEQ ID NO: 46 - protein, 17 aa, Mus musculus
YISSGSSSSFYVDTVKG

SEQ ID NO: 47 - protein, 7 aa, Mus musculus
GDRNFEV

SEQ ID NO: 48 - protein, 15 aa, Mus musculus
RASQSVSSSRYSYMH

SEQ ID NO: 49 - protein, 7 aa, Mus musculus
HASNLES

SEQ ID NO: 50 - protein, 9 aa, Mus musculus
QQSWEVPWT

SEQ ID NO: 51 - protein, 5 aa, Mus musculus
NYWMH

SEQ ID NO: 52 - protein, 17 aa, Mus musculus
YINPNTGYTDFNQKFKD

SEQ ID NO: 53 - protein, 8 aa, Mus musculus
QLGRNFDY

SEQ ID NO: 54 - protein, 15 aa, Mus musculus
RASQSVSSSRSTYIH

SEQ ID NO: 55 - protein, 7 aa, Mus musculus
YSSNLES

SEQ ID NO: 56 - protein, 9 aa, Mus musculus
HQSWEIPYT

SEQ ID NO: 57 - DNA, 348 bp, Artificial Sequence
  Synthetic
caagtgcaacttgtggaatctggaggaggagtggtgcaacctggaggatctcttagactttcttgcgcagcatctggatttacattcagcaatttcggcatacattgggtgagacaagcacctggaaagggcctagaatgggtggcatatatctcttctggaggatctgcagtgttctacgccgatacagtgaaaggaagatttacaatctctagagataactctaagaatacgctttatcttcaaatgaactctcttagagcagaagatacagcagtgtattattgcgcaaagagcgacagatatttcgactactgggggcagggaacaacagtgacagtgtcttct

SEQ ID NO: 58 - protein, 116 aa, Artificial Sequence
  Synthetic
QVQLVESGGGVVQPGGSLRLSCAASGFTFSNFGIHWVRQAPGKGLEWVAYISSGGSAVFYADTVKGRFTISRDNSKNTLYLQMNSLRAEDTAVYYCAKSDRYFDYWGQGTTVTVSS

SEQ ID NO: 59 - DNA, 333 bp, Artificial Sequence
  Synthetic
gaaatcgtgcttacacaatctcctgctactctaagtctgagtcctggagaaagagccaccctaagttgtagggcatctcaatctgtgtcttcttcttcttatagatatatccattggtatcaacagaagcccgggcaagcacctagacttcttatctactatgcatctaaccttgaatctggaatccctgcaagattcagcgggtctggatctggaacagatttcactttgacaatctcttctcttgaacctgaagatttcgccgtttattattgccaacattcttgggaaacaccttggacatttggacaaggaacaaagttagagatcaaa

SEQ ID NO: 60 - protein, 111 aa, Artificial Sequence
  Synthetic
EIVLTQSPATLSLSPGERATLSCRASQSVSSSSYRYIHWYQQKPGQAPRLLIYYASNLESGIPARFSGSGSGTDFTLTISSLEPEDFAVYYCQHSWETPWTFGQGTKLEIK

SEQ ID NO: 61 - protein, 443 aa, Artificial Sequence
  Synthetic
QVQLVESGGGVVQPGGSLRLSCAASGFTFSNFGIHWVRQAPGKGLEWVAYISSGGSAVFYADTVKGRFTISRDNSKNTLYLQMNSLRAEDTAVYYCAKSDRYFDYWGQGTTVTVSSASTKGPSVFPLAPCSRSTSESTAALGCLVKDYFPEPVTVSWNSGALTSGVHTFPAVLQSSGLYSLSSVVTVPSSSLGTKTYTCNVDHKPSNTKVDKRVESKYGPPCPPCPAPEFLGGPSVFLFPPKPKDTLMISRTPEVTCVVVDVSQEDPEVQFNWYVDGVEVHNAKTKPREEQFNSTYRVVSVLTVLHQDWLNGKEYKCKVSNKGLPSSIEKTISKAKGQPREPQVYTLPPSQEEMTKNQVSLTCLVKGFYPSDIAVEWESNGQPENNYKTTPPVLDSDGSFFLYSRLTVDKSRWQEGNVFSCSVLHEALHSHYTQKSLSLSLGK

SEQ ID NO: 62 - protein, 218 aa, Artificial Sequence
  Synthetic
EIVLTQSPATLSLSPGERATLSCRASQSVSSSSYRYIHWYQQKPGQAPRLLIYYASNLESGIPARFSGSGSGTDFTLTISSLEPEDFAVYYCQHSWETPWTFGQGTKLEIKRTVAAPSVFIFPPSDEQLKSGTASVVCLLNNFYPREAKVQWKVDNALQSGNSQESVTEQDSKDSTYSLSSTLTLSKADYEKHKVYACEVTHQGLSSPVTKSFNRGEC

SEQ ID NO: 63 - DNA, 342 bp, Artificial Sequence
  Synthetic
caagtgcagctgcaagagtctggccctggcctggtgaagccttctcagaccctgagcctgacctgcacagtgtctggctacagcatcacctctgactatgcctggaactggatcagacagcctcctggcaagggcctggagtggatgggctacatcagctactctggcagaacaagctacaaccctagcctgaagagcagactgaccatcagcagagacacaagcaagaatcagttcagcctgaagctgagctctgtgacagctgctgacacagctgtgtactactgtgctagacactatggagacttctggggccaaggcaccacagtgacagtgagcagc

SEQ ID NO: 64 - protein, 114 aa, Artificial Sequence
  Synthetic
QVQLQESGPGLVKPSQTLSLTCTVSGYSITSDYAWNWIRQPPGKGLEWMGYISYSGRTSYNPSLKSRLTISRDTSKNQFSLKLSSVTAADTAVYYCARHYGDFWGQGTTVTVSS

SEQ ID NO: 65 - DNA, 321 bp, Artificial Sequence
  Synthetic
gacattcagatgacacagagccctagcagcctgtctgcctctgtgggagacagagtgaccatcacctgcaaggcatctcagaatgtggacaccaatgtggcctggtatcagcagaagcctggcaaggcccctaagctgctgatctactctgcaagctacagatactctggagtgcctagcagattctctggctctggctctggcacagacttcaccctgaccatcagcagcctgcagcctgaggactttgccacctactactgtcagcagtacaacagctaccctagcacctttggccaaggcaccaagctggagatcaag

SEQ ID NO: 66 - protein, 107 aa, Artificial Sequence
  Synthetic
DIQMTQSPSSLSASVGDRVTITCKASQNVDTNVAWYQQKPGKAPKLLIYSASYRYSGVPSRFSGSGSGTDFTLTISSLQPEDFATYYCQQYNSYPSTFGQGTKLEIK

SEQ ID NO: 67 - protein, 441 aa, Artificial Sequence
  Synthetic
QVQLQESGPGLVKPSQTLSLTCTVSGYSITSDYAWNWIRQPPGKGLEWMGYISYSGRTSYNPSLKSRLTISRDTSKNQFSLKLSSVTAADTAVYYCARHYGDFWGQGTTVTVSSASTKGPSVFPLAPCSRSTSESTAALGCLVKDYFPEPVTVSWNSGALTSGVHTFPAVLQSSGLYSLSSVVTVPSSSLGTKTYTCNVDHKPSNTKVDKRVESKYGPPCPPCPAPEFLGGPSVFLFPPKPKDTLMISRTPEVTCVVVDVSQEDPEVQFNWYVDGVEVHNAKTKPREEQFNSTYRVVSVLTVLHQDWLNGKEYKCKVSNKGLPSSIEKTISKAKGQPREPQVYTLPPSQEEMTKNQVSLTCLVKGFYPSDIAVEWESNGQPENNYKTTPPVLDSDGSFFLYSRLTVDKSRWQEGNVFSCSVLHEALHSHYTQKSLSLSLGK

SEQ ID NO: 68 - protein, 214 aa, Artificial Sequence
  Synthetic
DIQMTQSPSSLSASVGDRVTITCKASQNVDTNVAWYQQKPGKAPKLLIYSASYRYSGVPSRFSGSGSGTDFTLTISSLQPEDFATYYCQQYNSYPSTFGQGTKLEIKRTVAAPSVFIFPPSDEQLKSGTASVVCLLNNFYPREAKVQWKVDNALQSGNSQESVTEQDSKDSTYSLSSTLTLSKADYEKHKVYACEVTHQGLSSPVTKSFNRGEC

SEQ ID NO: 69 - DNA, 348 bp, Artificial Sequence
  Synthetic
caagtgcaacttgtggaatctggaggaggagtggtgcaacctggaagatctcttagactttcttgcgcagcatctggatttacattcagttcgttcggcatgcattgggtgagacaagcacctggaaagggcctagaatgggtggcatatatctcttctggatcttcttcttctttctacgtcgatacagtgaaaggaagatttacaatctctagagataactctaagaatacgctttatcttcaaatgaactctcttagagcagaagatacagcagtgtattattgcgcaagaggagatagaaactttgaagtgtggggtcaggggacaacagtgacagtgtcttct

SEQ ID NO: 70 - protein, 116 aa, Artificial Sequence
  Synthetic
QVQLVESGGGVVQPGRSLRLSCAASGFTFSSFGMHWVRQAPGKGLEWVAYISSGSSSSFYVDTVKGRFTISRDNSKNTLYLQMNSLRAEDTAVYYCARGDRNFEVWGQGTTVTVSS

SEQ ID NO: 71 - DNA, 333 bp, Artificial Sequence
  Synthetic
gatatccagatgactcagagccctagcagcctgagcgccagcgtgggcgatagggtgactatcacttgtagggccagccagagcgtgagcagcagcaggtacagctacatgcactggttccagcagaagcctggcaaggctcctaagctgctgatctaccacgccagcaatctggagagcggcgtgcctagcaggttcagcggcagcggcagcggcactgatttcactctgactatcagcagcctgcagcctgaggatttcgccacttactactgtcagcagagctgggaggtgccttggactttcggccagggcactaagctggagatcaag

SEQ ID NO: 72 - protein, 111 aa, Artificial Sequence
  Synthetic
DIQMTQSPSSLSASVGDRVTITCRASQSVSSSRYSYMHWFQQKPGKAPKLLIYHASNLESGVPSRFSGSGSGTDFTLTISSLQPEDFATYYCQQSWEVPWTFGQGTKLEIK

SEQ ID NO: 73 - protein, 443 aa, Artificial Sequence
  Synthetic
QVQLVESGGGVVQPGRSLRLSCAASGFTFSSFGMHWVRQAPGKGLEWVAYISSGSSSSFYVDTVKGRFTISRDNSKNTLYLQMNSLRAEDTAVYYCARGDRNFEVWGQGTTVTVSSASTKGPSVFPLAPCSRSTSESTAALGCLVKDYFPEPVTVSWNSGALTSGVHTFPAVLQSSGLYSLSSVVTVPSSSLGTKTYTCNVDHKPSNTKVDKRVESKYGPPCPPCPAPEFLGGPSVFLFPPKPKDTLMISRTPEVTCVVVDVSQEDPEVQFNWYVDGVEVHNAKTKPREEQFNSTYRVVSVLTVLHQDWLNGKEYKCKVSNKGLPSSIEKTISKAKGQPREPQVYTLPPSQEEMTKNQVSLTCLVKGFYPSDIAVEWESNGQPENNYKTTPPVLDSDGSFFLYSRLTVDKSRWQEGNVFSCSVLHEALHSHYTQKSLSLSLGK

SEQ ID NO: 74 - protein, 218 aa, Artificial Sequence
  Synthetic
DIQMTQSPSSLSASVGDRVTITCRASQSVSSSRYSYMHWFQQKPGKAPKLLIYHASNLESGVPSRFSGSGSGTDFTLTISSLQPEDFATYYCQQSWEVPWTFGQGTKLEIKRTVAAPSVFIFPPSDEQLKSGTASVVCLLNNFYPREAKVQWKVDNALQSGNSQESVTEQDSKDSTYSLSSTLTLSKADYEKHKVYACEVTHQGLSSPVTKSFNRGEC

SEQ ID NO: 75 - DNA, 351 bp, Artificial Sequence
  Synthetic
caagtgcaacttgtgcaatctggagcagaagtgaagaagccaggtgcatctgtgaaagtgtcttgcaaagcatctggaaacacatttacaaactattggatgcattggatcagacaagcacctggacaaggacttgaatggatgggatacattaatcccaatacgggctacacggactttaaccagaaatttaaagatagagtaacacttacagcagataaatctacaagcacagcatatatggaactttcttctcttagatctgaagatacagcagtgtattattgcacacttcaacttggaagaaactttgattattggggccagggcacaacagtgacagtgtcttct

SEQ ID NO: 76 - protein, 117 aa, Artificial Sequence
  Synthetic
QVQLVQSGAEVKKPGASVKVSCKASGNTFTNYWMHWIRQAPGQGLEWMGYINPNTGYTDFNQKFKDRVTLTADKSTSTAYMELSSLRSEDTAVYYCTLQLGRNFDYWGQGTTVTVSS

SEQ ID NO: 77 - DNA, 333 bp, Artificial Sequence
  Synthetic
gatatccaaatgacacaatctccttcttctctttctgcatctgtgggagatagagtgacaatcacatgcagagcatctcaatctgtgtcttcttctagatctacatatatccattggtatcaacagaagccgggcaaggctccgaaactattgatctactattcttctaaccttgaatctggagtgccttctagattctcaggttctggatctggaacagatttcaccttaacaatctcttctcttcaacctgaagatttcgcgacgtattattgccatcaatcttgggaaatcccttatacatttggacaaggaacaaagttagagatcaaa

SEQ ID NO: 78 - protein, 111 aa, Artificial Sequence
  Synthetic
DIQMTQSPSSLSASVGDRVTITCRASQSVSSSRSTYIHWYQQKPGKAPKLLIYYSSNLESGVPSRFSGSGSGTDFTLTISSLQPEDFATYYCHQSWEIPYTFGQGTKLEIK

SEQ ID NO: 79 - protein, 444 aa, Artificial Sequence
  Synthetic
QVQLVQSGAEVKKPGASVKVSCKASGNTFTNYWMHWIRQAPGQGLEWMGYINPNTGYTDFNQKFKDRVTLTADKSTSTAYMELSSLRSEDTAVYYCTLQLGRNFDYWGQGTTVTVSSASTKGPSVFPLAPCSRSTSESTAALGCLVKDYFPEPVTVSWNSGALTSGVHTFPAVLQSSGLYSLSSVVTVPSSSLGTKTYTCNVDHKPSNTKVDKRVESKYGPPCPPCPAPEFLGGPSVFLFPPKPKDTLMISRTPEVTCVVVDVSQEDPEVQFNWYVDGVEVHNAKTKPREEQFNSTYRVVSVLTVLHQDWLNGKEYKCKVSNKGLPSSIEKTISKAKGQPREPQVYTLPPSQEEMTKNQVSLTCLVKGFYPSDIAVEWESNGQPENNYKTTPPVLDSDGSFFLYSRLTVDKSRWQEGNVFSCSVLHEALHSHYTQKSLSLSLGK

SEQ ID NO: 80 - protein, 218 aa, Artificial Sequence
  Synthetic
DIQMTQSPSSLSASVGDRVTITCRASQSVSSSRSTYIHWYQQKPGKAPKLLIYYSSNLESGVPSRFSGSGSGTDFTLTISSLQPEDFATYYCHQSWEIPYTFGQGTKLEIKRTVAAPSVFIFPPSDEQLKSGTASVVCLLNNFYPREAKVQWKVDNALQSGNSQESVTEQDSKDSTYSLSSTLTLSKADYEKHKVYACEVTHQGLSSPVTKSFNRGEC